European Patent Application EP 4 194 562 A1, published June 14, 2023. Title: Method for screening polypeptides acting on a target protein. Applicant: The National Institute of Advanced Industrial Science and Technology. The sequence listing filed with the application follows.

SEQUENCE LISTING (27 sequences)

SEQ ID NO: 1 - protein, 34 aa, Artificial Sequence
  synthetic peptide (library based on GTx1-15)
  misc_feature (5)..(6): Xaa can be any naturally occurring amino acid
  misc_feature (20)..(20): Xaa can be any naturally occurring amino acid
  misc_feature (29)..(29): Xaa can be any naturally occurring amino acid
  misc_feature (31)..(34): Xaa can be any naturally occurring amino acid
DCLGXXRKCIPDNDKCCRPXLVCSRTHKXCXXXX

SEQ ID NO: 2 - protein, 34 aa, Grammostola rosea
DCLGFMRKCIPDNDKCCRPNLVCSRTHKWCKYVF

SEQ ID NO: 3 - DNA, 2562 bp, Homo sapiens
atgacgaaacacggtagccgctcgactagctcgctgccgccggaaccgatggaaatcgtccgctctaaagcctgctcacgtcgtgttcgtctgaatgtgggcggacttgcccatgaagtcctgtggcggaccttagaccgcctgcctcgtacccgtttgggcaaattacgcgattgcaatacccacgattccctcttggaagtttgtgatgactactcattggatgataatgaatatttctttgatcggcatccgggtgccttcacatcgattctgaacttttaccgtacggggcgcctgcacatgatggaggaaatgtgcgctctgagctttagtcaggaactcgactattggggcattgacgaaatctaccttgaatcttgctgtcaagcgcgctatcaccagaaaaaagagcagatgaacgaagaacttaaacgcgaagcggaaacgctgcgcgaacgcgaaggtgaagaatttgacaacacctgttgcgcggaaaagcgcaagaaattgtgggatttgctggaaaagccgaactctagtgtcgcggcgaaaattctggccattatcagcattatgtttatcgtgttatcgactattgcactgtccctcaatacgttaccagaactgcaatcactcgatgagtttgggcaaagtaccgataatccgcagttggcccacgtggaagccgtatgcattgcgtggtttaccatggaatacttgttgcgctttctgagcagtcccaaaaaatggaaattcttcaaaggtccacttaacgcgattgatctgcttgccattctgccgtattacgttaccatcttcctgaccgagtcaaacaaatcggtgttgcagtttcaaaacgttcggcgcgtcgtccagattttccggattatgcgtattctgcgcattctgaaactggcccgtcattccaccgggcttcaaagcctgggctttacgctgcgtcgcagctataatgaactgggactcctgattctgtttctggcgatgggcatcatgatcttcagctcactcgtgttctttgcggagaaggatgaggatgatacgaaattcaaatccatcccggcaagcttttggtgggctacgattaccatgacgaccgtgggttacggtgacatttatccgaaaaccttgctgggcaaaatcgtcggtggcctttgctgtattgctggcgtgctggtcatcgcgctgccgattcccattattgtgaataacttctcagaattttacaaagaacagaagcgccaggagaaggccatcaaacgccgtgaagcgctggagcgcgctaaacgcaatggtagtattgtaagcatgaacatgaaagacgcatttgcgcgcagcatcgaaatgatggacatcgtagttgaaaagaatggggagaacatgggcaagaaagataaggtgcaggataaccatctgagcccaaacaaatggaagtggacgaaacgcactttatccgaaacctctagtagcaaatctttcgagactaaggaacagggatcaccggagaaagcccgctctagttcctccccacagcatctgaatgtgcaacagttagaagatatgtataacaaaatggccaaaactcaaagtcaacccattctgaataccaaagagagtgcagcacagtcgaaaccgaaagaagaactggagatggagtccatcccgtcgcctgtagcaccactgccgactcgtacggagggtgtgattgacatgcgttccatgagctctattgactcctttatcagctgtgcaaccgattttccggaagcaacgcgcttctctcactcccctctcacgtcgttaccgagtaaaacaggcggttcgaccgctccagaggttggctggcgtggtgccctgggtgccagcggaggacgtttcgtagaagcaaacccgagcccggacgcgagccagcatagctccttcttcatcgaatcaccgaaatcttcaatgaaaaccaacaatcccctcaaacttcgcgctctgaaagtgaacttcatggaaggggacccttctccactgttgccggttctggggatgtatcatgaccctttacgtaaccgtggctcggcagccgcggcggtagccggtcttgaatgtgccacactgttagataaagcggtcttatccccggaaagttcgatctatacaaccgctagcgcgaaaaccccgcctcggagcccagagaaacatactgctatcgcatttaactttgaagcaggcgttcatcagtacatcgatgcggataccgatgatgaaggccaactgctgtatagcgtggattcgagtccaccgaaaagtttacccggttcaacctcgccgaaattttccacaggcacccgtagcgaaaagaatcactttgagagcagtcctctcccgacatcgcctaaatttctgcgccagaattgcatttatagcacggaagcgctgactggcaagggtccgtctggccaggagaagtgtaaactggagaatcacatttctccggacgttcgtgtgctgcccggcggcggtgcgcatggctctacacgcgatcagtcaatt

SEQ ID NO: 4 - protein, 34 aa, Artificial Sequence
  synthetic peptide (Clone 4)
DCLGRRRKCIPDNDKCCRPLLVCSRTHKGCWVMG

SEQ ID NO: 5 - protein, 34 aa, Artificial Sequence
  synthetic peptide (Clone 9)
DCLGSSRKCIPDNDKCCRPPLVCSRTHKSCTLFL

SEQ ID NO: 6 - protein, 28 aa, Artificial Sequence
  synthetic peptide (Clone 16)
DCLGRWRKCIPDNDKCCRPILVLCTPSG

SEQ ID NO: 7 - protein, 34 aa, Artificial Sequence
  synthetic peptide (Clone 30)
DCLGPLRKCIPDTTNAVVQILYAVERTKKCWSAK

SEQ ID NO: 8 - protein, 34 aa, Artificial Sequence
  synthetic peptide (Clone 32)
DCLGSVRKCIPDNDKCCRPVLVCSRTHKFCFLVM

SEQ ID NO: 9 - protein, 34 aa, Artificial Sequence
  synthetic peptide (Clone 46)
DCLGYWRKCIPTTTNAVVQVLYAVERHKECIMAK

SEQ ID NO: 10 - protein, 34 aa, Artificial Sequence
  synthetic peptide (enriched (5 rounds) plasmid DNA sequence)
DCLGRWRKCIPDNDKCCRPILVLCTPSGLVPRGS

SEQ ID NO: 11 - protein, 34 aa, Artificial Sequence
  synthetic peptide (enriched (5 rounds) plasmid DNA sequence)
DCLGPPRKCIPDNDKCCRPVLVCSRTHKRCPTLV

SEQ ID NO: 12 - protein, 34 aa, Artificial Sequence; identical to SEQ ID NO: 4
  synthetic peptide (enriched (5 rounds) plasmid DNA sequence)

SEQ ID NO: 13 - protein, 34 aa, Artificial Sequence; identical to SEQ ID NO: 5
  synthetic peptide (enriched (5 rounds) plasmid DNA sequence)

SEQ ID NO: 14 - protein, 34 aa, Artificial Sequence
  synthetic peptide (enriched (5 rounds) plasmid DNA sequence)
DCLGGERKCIPDNDKCCRPPLVCSRTHKYCVVMI

SEQ ID NO: 15 - protein, 34 aa, Artificial Sequence
  synthetic peptide (enriched (5 rounds) plasmid DNA sequence)
DCLGALRKCIPDNDKCCRPVLVCSRTHKSCLLAK

SEQ ID NO: 16 - protein, 34 aa, Artificial Sequence
  synthetic peptide (enriched (5 rounds) plasmid DNA sequence)
DCLGEPRKCIPDNDKCCRPYLVCSRTHKMCMGII

SEQ ID NO: 17 - protein, 34 aa, Artificial Sequence; identical to SEQ ID NO: 7
  synthetic peptide (enriched (5 rounds) plasmid DNA sequence)

SEQ ID NO: 18 - protein, 34 aa, Artificial Sequence
  synthetic peptide (enriched (5 rounds) plasmid DNA sequence)
DCLGAFRKCIPDNDKCCRPILVCSRTHKTCIFYF

SEQ ID NO: 19 - protein, 34 aa, Artificial Sequence; identical to SEQ ID NO: 9
  synthetic peptide (enriched (5 rounds) plasmid DNA sequence)

SEQ ID NO: 20 - protein, 34 aa, Artificial Sequence
  synthetic peptide (enriched (5 rounds) plasmid DNA sequence)
DCLGMFRKCIPDKYCAYVILVPRGSSLSLSLAAA

SEQ ID NO: 21 - protein, 34 aa, Artificial Sequence
  synthetic peptide (enriched (5 rounds) plasmid DNA sequence)
DCLGMSRKCIPDNDKCCRPVLVCSRTHKMCILVK

SEQ ID NO: 22 - protein, 34 aa, Artificial Sequence
  synthetic peptide (enriched (5 rounds) plasmid DNA sequence)
DCLGHQRKCIPDNDKCCRPALVCSRTHKACTFVI

SEQ ID NO: 23 - protein, 34 aa, Artificial Sequence
  synthetic peptide (enriched (5 rounds) plasmid DNA sequence)
DCLGPARKCIPTTTNAVVQCLYAVERTKTVQVSD

SEQ ID NO: 24 - protein, 34 aa, Artificial Sequence
  synthetic peptide (enriched (5 rounds) plasmid DNA sequence)
DCLGTDRKCIPDNDKCCRPVLVCSRTHKMCIIAK

SEQ ID NO: 25 - protein, 34 aa, Artificial Sequence
  synthetic peptide (enriched (5 rounds) plasmid DNA sequence)
DCLGPLRKCIPDNDKCCRPILVCSRTHKFCIMAK

SEQ ID NO: 26 - protein, 34 aa, Artificial Sequence
  synthetic peptide (enriched (5 rounds) plasmid DNA sequence)
DCLGPPRKCIPTTTNAVVHTLYAVERTKNVLGFV

SEQ ID NO: 27 - protein, 34 aa, Artificial Sequence; identical to SEQ ID NO: 8
  synthetic peptide (enriched (5 rounds) plasmid DNA sequence)